European Patent Specification EP 3 858 388 B1, published July 3, 2024. Title: Chimeric Antigen Receptor (CAR) T Cells as Therapeutic Interventions for Auto- and Allo-Immunity. Applicant: Regents of the University of Minnesota. The sequence listing filed with the application follows.

SEQUENCE LISTING (1 sequence)

SEQ ID NO: 1 - DNA, 2538 bp, Artificial Sequence
  Synthetically generated construct
gccgccaccatgctgctgctggtgaccagcctgctgctgtgcgagctgccccaccccgcctttctgctgatccccgacatccagatgacccagaccacctccagcctgagcgccagcctgggcgaccgggtgaccatcagctgccgggccagccaggacatcagcaagtacctgaactggtatcagcagaagcccgacggcaccgtcaagctgctgatctaccacaccagccggctgcacagcggcgtgcccagccggtttagcggcagcggctccggcaccgactacagcctgaccatctccaacctggaacaggaagatatcgccacctacttttgccagcagggcaacacactgccctacacctttggcggcggaacaaagctggaaatcaccggcagcacctccggcagcggcaagcctggcagcggcgagggcagcaccaagggcgaggtgaagctgcaggaaagcggccctggcctggtggcccccagccagagcctgagcgtgacctgcaccgtgagcggcgtgagcctgcccgactacggcgtgagctggatccggcagccccccaggaagggcctggaatggctgggcgtgatctggggcagcgagaccacctactacaacagcgccctgaagagccggctgaccatcatcaaggacaacagcaagagccaggtgttcctgaagatgaacagcctgcagaccgacgacaccgccatctactactgcgccaagcactactactacggcggcagctacgccatggactactggggccagggcaccagcgtgaccgtgagcagcgaatctaagtacggaccgccctgccccccttgccctatgttctgggtgctggtggtggtcggaggcgtgctggcctgctacagcctgctggtcaccgtggccttcatcatcttttgggtgaaacggggcagaaagaaactcctgtatatattcaaacaaccatttatgagaccagtacaaactactcaagaggaagatggctgtagctgccgatttccagaagaagaagaaggaggatgtgaactgcgggtgaagttcagcagaagcgccgacgcccctgcctaccagcagggccagaatcagctgtacaacgagctgaacctgggcagaagggaagagtacgacgtcctggataagcggagaggccgggaccctgagatgggcggcaagcctcggcggaagaacccccaggaaggcctgtataacgaactgcagaaagacaagatggccgaggcctacagcgagatcggcatgaagggcgagcggaggcggggcaagggccacgacggcctgtatcagggcctgtccaccgccaccaaggatacctacgacgccctgcacatgcaggccctgcccccaaggctcgagggcggcggagagggcagaggaagtcttctaacatgcggtgacgtggaggagaatcccggccctaggatgcttctcctggtgacaagccttctgctctgtgagttaccacacccagcattcctcctgatcccacgcaaagtgtgtaacggaataggtattggtgaatttaaagactcactctccataaatgctacgaatattaaacacttcaaaaactgcacctccatcagtggcgatctccacatcctgccggtggcatttaggggtgactccttcacacatactcctcctctggatccacaggaactggatattctgaaaaccgtaaaggaaatcacagggtttttgctgattcaggcttggcctgaaaacaggacggacctccatgcctttgagaacctagaaatcatacgcggcaggaccaagcaacatggtcagttttctcttgcagtcgtcagcctgaacataacatccttgggattacgctccctcaaggagataagtgatggagatgtgataatttcaggaaacaaaaatttgtgctatgcaaatacaataaactggaaaaaactgtttgggacctccggtcagaaaaccaaaattataagcaacagaggtgaaaacagctgcaaggccacaggccaggtctgccatgccttgtgctcccccgagggctgctggggcccggagcccagggactgcgtctcttgccggaatgtcagccgaggcagggaatgcgtggacaagtgcaaccttctggagggtgagccaagggagtttgtggagaactctgagtgcatacagtgccacccagagtgcctgcctcaggccatgaacatcacctgcacaggacggggaccagacaactgtatccagtgtgcccactacattgacggcccccactgcgtcaagacctgcccggcaggagtcatgggagaaaacaacaccctggtctggaagtacgcagacgccggccatgtgtgccacctgtgccatccaaactgcacctacggatgcactgggccaggtcttgaaggctgtccaacgaatgggcctaagatcccgtccatcgccactgggatggtgggggccctcctcttgctgctggtggtggccctggggatcggcctcttcatgtga